European Patent Application EP 4 137 794 A1, published February 22, 2023. Title: Cyanine dyes and their usage for in vivo staining of microorganisms and other living cells. Applicant: Philipps-Universität Marburg. Application EP EP 21 192 451.9, filed August 16, 2022. The sequence listing filed with the application follows.

SEQUENCE LISTING (4 sequences)

SEQ ID NO: 1 - protein, 5 aa, synthetic construct
  REGION 1..5: note = A is L-cyclohexylalanine; R is D-arginine
CARAR

SEQ ID NO: 2 - protein, 4 aa, synthetic construct
  REGION 1..4: note = A is L-cyclohexylalanine; R is D-arginine
ARAR

SEQ ID NO: 3 - protein, 6 aa, synthetic construct
  REGION 1..6: note = A is L-cyclohexylalanine; R is D-arginine
RARARA

SEQ ID NO: 4 - protein, 6 aa, synthetic construct
  REGION 1..6: note = A is L-cyclohexylalanine; R is D-arginine
RFRFRF